European Patent Application EP 4 116 428 A1, published January 11, 2023. Title: BLOCK COPOLYMER AND METHOD FOR PRODUCING SAME. Applicant: NATIONAL UNIVERSITY CORPORATION HOKKAIDO UNIVERSITY. Application EP21760911.4. The sequence listing filed with the application follows.

SEQUENCE LISTING (3 sequences)

SEQ ID NO: 1 - protein, 517 aa, Megasphaera elsdenii
MRKVEIITAEQAAQLVKDNDTITSIGFVSSAHPEALTKALEKRFLDTNTPQNLTYIYAGSQGKRDGRAAEHLAHTGLLKRAIIGHWQTVPAIGKLAVENKIEAYNFSQGTLVHWFRALAGHKLGVFTDIGLETFLDPRQLGGKLNDVTKEDLVKLIEVDGHEQLFYPTFPVNVAFLRGTYADESGNITMDEEIGPFESTSVAQAVHNCGGKVVVQVKDVVAHGSLDPRMVKIPGIYVDYVVVAAPEDHQQTYDCEYDPSLSGEHRAPEGAADAALPMSAKKIIGRRGALELTENAVVNLGVGAPEYVASVAGEEGIADTITLTVEGGAIGGVPQGGARFGSSRNADAIIDHTYQFDFYDGGGLDIAYLGLAQCDGSGNINVSKFGTNVAGCGGFPNISQQTPNVYFCGTFTAGGLKIAVEDGKVKILQEGKAKKFIKAVDQITFNGSYAARNGKHVLYITERCVFELTKEGLKLIEVAPGIDIEKDILAHMDFKPIIDNPKLMDARLFQDGPMGLKK

SEQ ID NO: 2 - protein, 560 aa, Pseudomonas putida
MLQTRIIKPAEGAYAYPLLIKRLLMSGSRYEKTREIVYRDQMRLTYPQLNERIARLANVLTEAGVKAGDTVAVMDWDSHRYLECMFAIPMIGAVVHTINVRLSPEQILYTMNHAEDRVVLVNSDFVGLYQAIAGQLTTVDKTLLLTDGPDKTAELPGLVGEYEQLLAAASPRYDFPDFDENSVATTFYTTGTTGNPKGVYFSHRQLVLHTLAEASVTGSIDSVRLLGSNDVYMPITPMFHVHAWGIPYAATMLGMKQVYPGRYEPDMLVKLWREEKVTFSHCVPTILQMLLNCPNAQGQDFGGWKIIIGGSSLNRSLYQAALARGIQLTAAYGMSETCPLISAAHLNDELQAGSEDERVTYRIKAGVPVPLVEAAIVDGEGNFLPADGETQGELVLRAPWLTMGYFKEPEKSEELWQGGWLHTGDVATLDGMGYIDIRDRIKDVIKTGGEWVSSLDLEDLISRHPAVREVAVVGVADPQWGERPFALLVARDGHDIDAKALKEHLKPFVEQGHINKWAIPSQIALVTEIPKTSVGKLDKKRIRQDIVQWQASNSAFLSTL

SEQ ID NO: 3 - protein, 585 aa, Artificial Sequence
  PhaCAR
MSQPSYGPLFEALAHYNDKLLAMAKAQTERTAQALLQTNLDDLGQVLEQGSQQPWQLIQAQMNWWQDQLKLMQHTLLKSAGQPSEPVITPERSDRRFKAEAWSEQPIYDYLKQSYLLTARHLLASVDALEGVPQKSRERLRFFTRQYVNAMAPANFLATNPEAQRLLIESGGESLRAGVRNMMEDLTRGKISQTDESAFEVGRNVAVTEGAVVFENEYFQLLQYKPLTDKVHARPLLMVPPCINKYYILDLQPESSLVRHVVEQGHTVFLVSWRNPDASMAGSTWDDYIEHAAIRAIEVARDISGQDKINVLGFCVGGTIVSTALAVLAARGEHPAASVTLLTTLLDFADTGILDVFVDEGHVQLREATLGGGAGAPCALLRGLELANTFSFLRPNDLVWNYVVDNYLKGNTPVPFDLLFWNGDATNLPGPWYCWYLRHTYLQNELKVPGKLTVCGVPVDLASIDVPTYIYGSREDHIVPWTAAYASTALLANKLRFVLGASGHIAGVINPPAKNKRSHWTNDALPESPQQWLAGAIEHHGSWWPDWTAWLAGQAGAKRAAPANYGNARYRAIEPAPGRYVKAKA